European Patent Specification EP 4 045 681 B1, published July 16, 2025. Title: DETERMINATION OF NUCLEIC ACID SEQUENCE CONCENTRATIONS. Applicant: STILLA TECHNOLOGIES ANDRÉ Barbara DANGLA Rémi. The sequence listing filed with the application follows.

SEQUENCE LISTING (9 sequences)

SEQ ID NO: 1 - DNA, 30 bp, Artificial Sequence
  BRAF V600 WT - Primer Forward
tactgttttcctttacttactacacctcag

SEQ ID NO: 2 - DNA, 21 bp, Artificial Sequence
  BRAF V600 WT - Primer Reverse
actgatgggacccactccatc

SEQ ID NO: 3 - DNA, 20 bp, Artificial Sequence
  BRAF V600 WT - Probe (FAM)
  modified_base 10: /mod_base="OTHER" /note="Locked Nucleic Acid (LAN) base"
  modified_base 11: /mod_base="OTHER" /note="Locked Nucleic Acid (LAN) base"
ctagctacagtgaaatctcg

SEQ ID NO: 4 - DNA, 23 bp, Artificial Sequence
  EGFR L858 WT - Primer Forward
gcagcatgtcaagatcacagatt

SEQ ID NO: 5 - DNA, 25 bp, Artificial Sequence
  EGFR L858 WT - Primer Reverse
cctccttctgcatggtattctttct

SEQ ID NO: 6 - DNA, 16 bp, Artificial Sequence
  EGFR L858 WT - Probe (HEX)
  modified_base 8: /mod_base="OTHER" /note="Locked Nucleic Acid (LAN) base"
  modified_base 9: /mod_base="OTHER" /note="Locked Nucleic Acid (LAN) base"
  modified_base 11: /mod_base="OTHER" /note="Locked Nucleic Acid (LAN) base"
agtttggccagcccaa

SEQ ID NO: 7 - DNA, 25 bp, Artificial Sequence
  ALB - Primer Forward
tgaaacatacgttcccaaagagttt

SEQ ID NO: 8 - DNA, 26 bp, Artificial Sequence
  ALB - Primer Reverse
ctctccttctcagaaagtgtgcatat

SEQ ID NO: 9 - DNA, 25 bp, Artificial Sequence
  ALB - Probe (Cy5)
tgctgaaacattcaccttccatgca